European Patent Application EP 4 428 528 A2, published September 11, 2024. Title: LABELED NUCLEOTIDE COMPOSITIONS AND METHODS FOR NUCLEIC ACID SEQUENCING. Applicant: Quantum-Si Incorporated. The sequence listing filed with the application follows.

SEQUENCE LISTING (10 sequences)

SEQ ID NO: 1 - DNA, 253 bp, synthetic construct
  misc_feature 1..253: note = Synthetic Polynucleotide
  source 1..253: mol_type = other DNA
aacccaccccccaaacacaacataatctctaatcacaacaaccaacaccaacaccaccaaacaaacatatctctctcaacaaacacaaccaccccaacacaaacacatacctctccaacaacaacaaaccacacactaaaacacacacatacatctctcaacaacaacaacccaacaccaccaaaaaacacaatatctcttctcacaacaacaaaccccaatcaaaaaaaacacacatattctctctcaacaa

SEQ ID NO: 2 - DNA, 266 bp, synthetic construct
  misc_feature 1..266: note = Synthetic Polynucleotide
  source 1..266: mol_type = other DNA
aacccaccaccaccaaaacacacacatatctctctcaacaacaacaacccaccaccaccaaaacacacacatatctctctcaacaacaacaacccaccaccaccaaaacacacacatatctctctcaacaacaacaacccaccaccaccaaaacacacacatatctctctcaacaacaacaacccaccaccaccaaaacacacacatatctctctcaacaacaacaacccaccaccaccaaaacacacacatatctctctcaacaa

SEQ ID NO: 3 - DNA, 219 bp, synthetic construct
  misc_feature 1..219: note = Synthetic Polynucleotide
  source 1..219: mol_type = other DNA
acaccaacaataaaaaaaaaaaacctctccaaacacaacacaaaaaaaaaaaaaaatactcccaacaacaaacaaaaaaaaaaaaaaaaaaaaaaaaaaaatatctctcacaacaacaacaaaaaaaaaaaaaaatatccctctcaacacacaacaataaaaaaaaaaaatctcctcacaacaaaacaaaaaaaaaaaaaaaaaaatttctctaaacac

SEQ ID NO: 4 - DNA, 263 bp, synthetic construct
  misc_feature 1..263: note = Synthetic Polynucleotide
  source 1..263: mol_type = other DNA
aaaaaaaaaaaaaaaaaaaaaatatctctctcaacaacaacaacaaaaaaaaaaaaaaaaaaaaaaatatctctctcaacaacaacaacaaaaaaaaaaaaaaaaaaaaaaatatctctctcaacaacaacaacaaaaaaaaaaaaaaaaaaaaaaatatctctctcaacaacaacaacaaaaaaaaaaaaaaaaaaaaaaatatctctctcaacaacaacaacaaaaaaaaaaaaaaaaaaaaaaatatctctctcaacaac

SEQ ID NO: 5 - DNA, 20 bp, synthetic construct
  misc_feature 1..20: note = Synthetic Polynucleotide
  source 1..20: mol_type = other DNA
ccacgcgtggaacacttgtg

SEQ ID NO: 6 - DNA, 45 bp, synthetic construct
  misc_feature 1..45: note = Synthetic Polynucleotide
  misc_feature 8..9: note = Modified by iCy3
  source 1..45: mol_type = other DNA
cacaagccggttccaggcaggcgttcgcctgtgttccacgcgtgg

SEQ ID NO: 7 - DNA, 53 bp, synthetic construct
  misc_feature 1..53: note = Synthetic Polynucleotide
  misc_feature 53: note = Modified by a luminescent label
  source 1..53: mol_type = other DNA
cccgcagcgcgcgtacacttgtgtcgcttgcgcccttgggacgcgccaccgtc

SEQ ID NO: 8 - DNA, 53 bp, synthetic construct
  misc_feature 1..53: note = Synthetic Polynucleotide
  source 1..53: mol_type = other DNA
gacggtggcgcgtacacttgtgtcgcttgcgcccttgggacgcgcgctgcggg

SEQ ID NO: 9 - DNA, 90 bp, synthetic construct
  misc_feature 1..90: note = Synthetic Polynucleotide
  misc_feature 47..48: note = Modified by iCy3
  misc_feature 50..51: note = Modified by iCy3
  source 1..90: mol_type = other DNA
ccacgcctggaacccttgggcctggtccttggaccagcgatgctttaagctcgggtactgttcagtaccgcccaagggttccaggcgtgg

SEQ ID NO: 10 - DNA, 10 bp, synthetic construct
  misc_feature 1..10: note = Synthetic Polynucleotide
  source 1..10: mol_type = other DNA
tccgtacgac